European Patent Specification EP 3 595 702 B1, published April 26, 2023. Title: Modified Globin Proteins. The sequence listing filed with the application follows.

SEQUENCE LISTING (18 sequences)

SEQ ID NO: 1 - protein, 146 aa, Homo sapiens
VHLTPEEKSAVTALWGKVNVDEVGGEALGRLLVVYPWTQRFFESFGDLSTPDAVMGNPKVKAHGKKVLGAFSDGLAHLDNLKGTFATLSELHCDKLHVDPENFRLLGNVLVCVLAHHFGKEFTPPVQAAYQKVVAGVANALAHKYH

SEQ ID NO: 2 - protein, 141 aa, Homo sapiens
VLSPADKTNVKAAWGKVGAHAGEYGAEALERMFLSFPTTKTYFPHFDLSHGSAQVKGHGKKVADALTNAVAHVDDMPNALSALSDLHAHKLRVDPVNFKLLSHCLLVTLAAHLPAEFTPAVHASLDKFLASVSTVLTSKYR

SEQ ID NO: 3 - protein, 146 aa, Homo sapiens
GHFTEEDKATITSLWGKVNVEDAGGETLGRLLVVYPWTQRFFDSFGNLSSASAIMGNPKVKAHGKKVLTSLGDAIKHLDDLKGTFAQLSELHCDKLHVDPENFKLLGNVLVTVLAIHFGKEFTPEVQASWQKMVTAVASALSSRYH

SEQ ID NO: 4 - protein, 146 aa, Homo sapiens
GHFTEEDKATITSLWGKVNVEDAGGETLGRLLVVYPWTQRFFDSFGNLSSASAIMGNPKVKAHGKKVLTSLGDAIKHLDDLKGTFAQLSELHCDKLHVDPENFKLLGNVLVTVLAIHFGKEFTPEVQASWQKMVTGVASALSSRYH

SEQ ID NO: 5 - protein, 146 aa, Artificial Sequence
  βV1M (reference protein)
MHLTPEEKSAVTALWGKVNVDEVGGEALGRLLVVYPWTQRFFESFGDLSTPDAVMGNPKVKAHGKKVLGAFSDGLAHLDNLKGTFATLSELHCDKLHVDPENFRLLGNVLVCVLAHHFGKEFTPPVQAAYQKVVAGVANALAHKYH

SEQ ID NO: 6 - protein, 141 aa, Artificial Sequence
  αV1M mutant (reference protein)
MLSPADKTNVKAAWGKVGAHAGEYGAEALERMFLSFPTTKTYFPHFDLSHGSAQVKGHGKKVADALTNAVAHVDDMPNALSALSDLHAHKLRVDPVNFKLLSHCLLVTLAAHLPAEFTPAVHASLDKFLASVSTVLTSKYR

SEQ ID NO: 7 - protein, 146 aa, Artificial Sequence
  γ1G1M (reference protein)
MHFTEEDKATITSLWGKVNVEDAGGETLGRLLVVYPWTQRFFDSFGNLSSASAIMGNPKVKAHGKKVLTSLGDAIKHLDDLKGTFAQLSELHCDKLHVDPENFKLLGNVLVTVLAIHFGKEFTPEVQASWQKMVTAVASALSSRYH

SEQ ID NO: 8 - protein, 146 aa, Artificial Sequence
  γ2G1M (reference protein)
MHFTEEDKATITSLWGKVNVEDAGGETLGRLLVVYPWTQRFFDSFGNLSSASAIMGNPKVKAHGKKVLTSLGDAIKHLDDLKGTFAQLSELHCDKLHVDPENFKLLGNVLVTVLAIHFGKEFTPEVQASWQKMVTGVASALSSRYH

SEQ ID NO: 9 - protein, 146 aa, Artificial Sequence
  βT84Y modified haemoglobin subunit
VHLTPEEKSAVTALWGKVNVDEVGGEALGRLLVVYPWTQRFFESFGDLSTPDAVMGNPKVKAHGKKVLGAFSDGLAHLDNLKGYFATLSELHCDKLHVDPENFRLLGNVLVCVLAHHFGKEFTPPVQAAYQKVVAGVANALAHKYH

SEQ ID NO: 10 - protein, 146 aa, Artificial Sequence
  βT84Y modified haemoglobin subunit (V1M mutant)
MHLTPEEKSAVTALWGKVNVDEVGGEALGRLLVVYPWTQRFFESFGDLSTPDAVMGNPKVKAHGKKVLGAFSDGLAHLDNLKGYFATLSELHCDKLHVDPENFRLLGNVLVCVLAHHFGKEFTPPVQAAYQKVVAGVANALAHKYH

SEQ ID NO: 11 - protein, 141 aa, Artificial Sequence
  αL91Y modified haemoglobin subunit (V1M mutant)
MLSPADKTNVKAAWGKVGAHAGEYGAEALERMFLSFPTTKTYFPHFDLSHGSAQVKGHGKKVADALTNAVAHVDDMPNALSALSDLHAHKYRVDPVNFKLLSHCLLVTLAAHLPAEFTPAVHASLDKFLASVSTVLTSKYR

SEQ ID NO: 12 - protein, 141 aa, Artificial Sequence
  αL91Y modified haemoglobin subunit
VLSPADKTNVKAAWGKVGAHAGEYGAEALERMFLSFPTTKTYFPHFDLSHGSAQVKGHGKKVADALTNAVAHVDDMPNALSALSDLHAHKYRVDPVNFKLLSHCLLVTLAAHLPAEFTPAVHASLDKFLASVSTVLTSKYR

SEQ ID NO: 13 - protein, 146 aa, Artificial Sequence
  γ2L96Y modified haemoglobin subunit (G1M Mutant)
MHFTEEDKATITSLWGKVNVEDAGGETLGRLLVVYPWTQRFFDSFGNLSSASAIMGNPKVKAHGKKVLTSLGDAIKHLDDLKGTFAQLSELHCDKYHVDPENFKLLGNVLVTVLAIHFGKEFTPEVQASWQKMVTGVASALSSRYH

SEQ ID NO: 14 - protein, 141 aa, Artificial Sequence
  αL29F modified haemoglobin subunit (V1M mutant)
MLSPADKTNVKAAWGKVGAHAGEYGAEAFERMFLSFPTTKTYFPHFDLSHGSAQVKGHGKKVADALTNAVAHVDDMPNALSALSDLHAHKLRVDPVNFKLLSHCLLVTLAAHLPAEFTPAVHASLDKFLASVSTVLTSKYR

SEQ ID NO: 15 - protein, 146 aa, Artificial Sequence
  γ2V67F modified haemoglobin subunit (G1M Mutant)
MHFTEEDKATITSLWGKVNVEDAGGETLGRLLVVYPWTQRFFDSFGNLSSASAIMGNPKVKAHGKKFLTSLGDAIKHLDDLKGTFAQLSELHCDKLHVDPENFKLLGNVLVTVLAIHFGKEFTPEVQASWQKMVTGVASALSSRYH

SEQ ID NO: 16 - protein, 141 aa, Artificial Sequence
  αL29F and αL91Y modified haemoglobin subunit (V1M mutant)
MLSPADKTNVKAAWGKVGAHAGEYGAEAFERMFLSFPTTKTYFPHFDLSHGSAQVKGHGKKVADALTNAVAHVDDMPNALSALSDLHAHKYRVDPVNFKLLSHCLLVTLAAHLPAEFTPAVHASLDKFLASVSTVLTSKYR

SEQ ID NO: 17 - protein, 146 aa, Artificial Sequence
  γ2V67F and γ2L96Y modified haemoglobin subunit (G1M Mutant)
MHFTEEDKATITSLWGKVNVEDAGGETLGRLLVVYPWTQRFFDSFGNLSSASAIMGNPKVKAHGKKFLTSLGDAIKHLDDLKGTFAQLSELHCDKYHVDPENFKLLGNVLVTVLAIHFGKEFTPEVQASWQKMVTGVASALSSRYH

SEQ ID NO: 18 - protein, 153 aa, Artificial Sequence
  Human myoglobin
GLSDGEWQLVLNVWGKVEADIPGHGQEVLIRLFKGHPETLEKFDKFKHLKSEDEMKASEDLKKHGATVLTALGGILKKKGHHEAEIKPLAQSHATKHKIPVKYLEFISECIIQVLQSKHPGDFGADAQGAMNKALELFRKDMASNYKELGFQG